European Patent Application EP 4 218 743 A2, published August 2, 2023. Title: OLEUROPEIN FOR USE IN CARTILAGE BREAKDOWN. Applicant: Société des Produits Nestlé S.A. Application EP 23155898.2, filed May 28, 2014. The sequence listing filed with the application follows.

SEQUENCE LISTING (8 sequences)

SEQ ID NO: 1 - DNA, 23 bp, Bos taurus
  source 1..23: mol_type = genomic DNA
aagggcattctaggctacactga

SEQ ID NO: 2 - DNA, 24 bp, Bos taurus
  source 1..24: mol_type = genomic DNA
agagtgagtgtcgctgttgaagtc

SEQ ID NO: 3 - DNA, 20 bp, Bos taurus
  source 1..20: mol_type = genomic DNA
cacctcagccaccatcacag

SEQ ID NO: 4 - DNA, 20 bp, Bos taurus
  source 1..20: mol_type = genomic DNA
agtactctggcccgaaggtc

SEQ ID NO: 5 - DNA, 24 bp, Bos taurus
  source 1..24: mol_type = genomic DNA
cacccatcaatttttcaagacaga

SEQ ID NO: 6 - DNA, 19 bp, Bos taurus
  source 1..19: mol_type = genomic DNA
ccaccccatggttctttcc

SEQ ID NO: 7 - DNA, 28 bp, Bos taurus
  source 1..28: mol_type = genomic DNA
gcagagagctacctgaaatcatactact

SEQ ID NO: 8 - DNA, 23 bp, Bos taurus
  source 1..23: mol_type = genomic DNA
aatcacagagcttgctgcagttt